European Patent Specification EP 2 780 360 B1, published March 8, 2023. Title: COMPOSITIONS AND METHODS FOR TREATING AUTOIMMUNE AND INFLAMMATORY DISORDERS. Applicant: SANFORD-BURNHAM MEDICAL RESEARCH INSTITUTE WARE, Carl F. SEDY, John. The sequence listing filed with the application follows.

SEQUENCE LISTING (82 sequences)

SEQ ID NO: 1 - DNA, 28 bp, Artificial Sequence
  Primer
agtcagatctgcgtgcaggatgctgttg

SEQ ID NO: 2 - DNA, 30 bp, Artificial Sequence
  Primer
agtcctcgagggcttacaaagcttgaaggg

SEQ ID NO: 3 - DNA, 31 bp, Artificial Sequence
  Primer
agtcagatctgtgcaggaaatgaagacattg

SEQ ID NO: 4 - DNA, 36 bp, Artificial Sequence
  Primer
agtcctcgagtcagaaacagacttaactcctcacac

SEQ ID NO: 5 - DNA, 28 bp, Artificial Sequence
  Primer
agctagatctgcgtgcaggatgctgatg

SEQ ID NO: 6 - DNA, 34 bp, Artificial Sequence
  Primer
agtcctcgagaaggcttacaaagcttgaaggacc

SEQ ID NO: 7 - DNA, 32 bp, Artificial Sequence
  Primer
aaacccgaagcagtgcaattaggaaatcagtg

SEQ ID NO: 8 - DNA, 32 bp, Artificial Sequence
  Primer
taattgcactgcttcgggtttgcatatttcag

SEQ ID NO: 9 - DNA, 34 bp, Artificial Sequence
  Primer
ttaggaaatgcgtgttgtcccccatgtaaacaag

SEQ ID NO: 10 - DNA, 33 bp, Artificial Sequence
  Primer
gggacaacacgcatttcctaattgcacttcttc

SEQ ID NO: 11 - DNA, 34 bp, Artificial Sequence
  Primer
cagtgttgtgccccatgtaaacaaggatatcgtg

SEQ ID NO: 12 - DNA, 33 bp, Artificial Sequence
  Primer
tttacatggggcacaacactgatttcctaattg

SEQ ID NO: 13 - DNA, 35 bp, Artificial Sequence
  Primer
tgtaaacaagcatatcgtgttacaggacaatgtac

SEQ ID NO: 14 - DNA, 36 bp, Artificial Sequence
  Primer
aacacgatatgcttgtttacatgggggacaacactg

SEQ ID NO: 15 - DNA, 38 bp, Artificial Sequence
  Primer
cccccatgtaaacaaggagctcgtgttacaggacaatg

SEQ ID NO: 16 - DNA, 38 bp, Artificial Sequence
  Primer
cattgtcctgtaacacgagctccttgtttacatggggg

SEQ ID NO: 17 - DNA, 38 bp, Artificial Sequence
  Primer
caaggatatgctgttacaggacaatgtacgcaatatac

SEQ ID NO: 18 - DNA, 33 bp, Artificial Sequence
  Primer
tcctgtaacagcatatccttgtttacatggggg

SEQ ID NO: 19 - DNA, 33 bp, Artificial Sequence
  Primer
tatcgtgttgcaggacaatgtacgcaatatacg

SEQ ID NO: 20 - DNA, 36 bp, Artificial Sequence
  Primer
acattgtcctgcaacacgatatccttgtttacatgg

SEQ ID NO: 21 - DNA, 35 bp, Artificial Sequence
  Primer
cgtgttacagcacaatgtacgcaatatacgagtac

SEQ ID NO: 22 - DNA, 35 bp, Artificial Sequence
  Primer
cgtacattgtgctgtaacacgatatccttgtttac

SEQ ID NO: 23 - DNA, 45 bp, Artificial Sequence
  Primer
aaacaaggatatcgtgttacaaaacaatgtacgcaatatacgagt

SEQ ID NO: 24 - DNA, 45 bp, Artificial Sequence
  Primer
actcgtatattgcgtacattgttttgtaacacgatatccttgttt

SEQ ID NO: 25 - DNA, 34 bp, Artificial Sequence
  Primer
caatgtacggcatatacgagtacaacatgtacag

SEQ ID NO: 26 - DNA, 38 bp, Artificial Sequence
  Primer
actcgtatatgccgtacattgtcctgtaacacgatatc

SEQ ID NO: 27 - DNA, 35 bp, Artificial Sequence
  Primer
acgcaatatgcgagtacaacatgtacactttgccc

SEQ ID NO: 28 - DNA, 36 bp, Artificial Sequence
  Primer
tgttgtactcgcatattgcgtacattgttctgtaac

SEQ ID NO: 29 - DNA, 34 bp, Artificial Sequence
  Primer
gtatcaggggcttacaattgtaccaattgcactg

SEQ ID NO: 30 - DNA, 35 bp, Artificial Sequence
  Primer
acaattgtaagcccctgatacatacgtaccgttag

SEQ ID NO: 31 - DNA, 35 bp, Artificial Sequence
  Primer
ttttccgttgcaggcgtccaacatcacaagcaacg

SEQ ID NO: 32 - DNA, 34 bp, Artificial Sequence
  Primer
ttggacgcctgcaacggaaaatgacgtataattc

SEQ ID NO: 33 - DNA, 43 bp, Artificial Sequence
  Primer
catgtgatgtagcgctttatataaagagacaatctgaacactc

SEQ ID NO: 34 - DNA, 39 bp, Artificial Sequence
  Primer
ctttatataaagcgctacatcacatgattctttcccatg

SEQ ID NO: 35 - DNA, 43 bp, Artificial Sequence
  Primer
atgtgatgtacagcattatataaagagacaatctgaacactcc

SEQ ID NO: 36 - DNA, 41 bp, Artificial Sequence
  Primer
ttgtctctttatataatgctgtacatcacatgattctttcc

SEQ ID NO: 37 - DNA, 38 bp, Artificial Sequence
  Primer
ctttatataaaggaccaatctgaacactccatcttagc

SEQ ID NO: 38 - DNA, 45 bp, Artificial Sequence
  Primer
gtgttcagattggtcctttatataaagctgtacatcacatgattc

SEQ ID NO: 39 - DNA, 37 bp, Artificial Sequence
  Primer
agagacaatctgcacactccatcttagcaggagatcc

SEQ ID NO: 40 - DNA, 41 bp, Artificial Sequence
  Primer
aagatggagtgtggagattgtctctttatataaagctgtac

SEQ ID NO: 41 - DNA, 37 bp, Artificial Sequence
  Primer
ctttgaactagcatgccctgtgaaatactgtgctaac

SEQ ID NO: 42 - DNA, 38 bp, Artificial Sequence
  Primer
tcacagggcatgctagttcaaagggatctcctgctaag

SEQ ID NO: 43 - DNA, 37 bp, Artificial Sequence
  Primer
gaactagaatgcgctgtgaaatactgtgctaacaggc

SEQ ID NO: 44 - DNA, 35 bp, Artificial Sequence
  Primer
gtatttcacagcgcattctagttcaaagggatctc

SEQ ID NO: 45 - DNA, 40 bp, Artificial Sequence
  Primer
acaagttgggcggaagagaagaacatttcatttttcattc

SEQ ID NO: 46 - DNA, 42 bp, Artificial Sequence
  Primer
cttctcttccgcccaacttgtttgtctatcttcaagttttac

SEQ ID NO: 47 - DNA, 36 bp, Artificial Sequence
  Primer
tgttctgcaaattttcagtctaatctcattgaaagc

SEQ ID NO: 48 - DNA, 37 bp, Artificial Sequence
  Primer
gattagactgaaaatttgcagaacagcggtatgaccc

SEQ ID NO: 49 - DNA, 38 bp, Artificial Sequence
  Primer
gctgttctgcattttttcagtctaatctcattgaaagc

SEQ ID NO: 50 - DNA, 32 bp, Artificial Sequence
  Primer
tagactgaaaaaatgcagaacagcggtatgac

SEQ ID NO: 51 - DNA, 38 bp, Artificial Sequence
  Primer
gttctgcaaatgctcagtctaatctcattgaaagccac

SEQ ID NO: 52 - DNA, 35 bp, Artificial Sequence
  Primer
gagattagactgagcatttgcagaacagcggtatg

SEQ ID NO: 53 - DNA, 37 bp, Artificial Sequence
  Primer
caaattttcagcataatctcattgaaagccactcaac

SEQ ID NO: 54 - DNA, 34 bp, Artificial Sequence
  Primer
caatgagattatgctgaaaatttgcagaacagcg

SEQ ID NO: 55 - DNA, 38 bp, Artificial Sequence
  Primer
cattgaaagcgactcaacaactctttatgtgacagatg

SEQ ID NO: 56 - DNA, 40 bp, Artificial Sequence
  Primer
gttgttgagtcgctttcaatgagattagactgaaaatttg

SEQ ID NO: 57 - DNA, 42 bp, Artificial Sequence
  Primer
tgaaagccaccatacaactctttatgtgacagatgtaaaaag

SEQ ID NO: 58 - DNA, 36 bp, Artificial Sequence
  Primer
aagagttgtatggtggctttcaatgagattagactg

SEQ ID NO: 59 - DNA, 18 bp, Artificial Sequence
  Primer
actaccgcccagcagtgt

SEQ ID NO: 60 - DNA, 19 bp, Artificial Sequence
  Primer
gtgtcatggggagaaccaa

SEQ ID NO: 61 - DNA, 18 bp, Artificial Sequence
  Primer
ggcggtgcctatcactgt

SEQ ID NO: 62 - DNA, 20 bp, Artificial Sequence
  Primer
ttctgaaaccccagtccttg

SEQ ID NO: 63 - DNA, 20 bp, Artificial Sequence
  Primer
tctcttgctgttgctgatgg

SEQ ID NO: 64 - DNA, 20 bp, Artificial Sequence
  Primer
ctcgtgagaccttcgctctt

SEQ ID NO: 65 - DNA, 21 bp, Artificial Sequence
  Primer
cagcctcttctccttcctgat

SEQ ID NO: 66 - DNA, 20 bp, Artificial Sequence
  Primer
gccagagggctgattagaga

SEQ ID NO: 67 - DNA, 21 bp, Artificial Sequence
  Primer
agcagctccccactgggtatg

SEQ ID NO: 68 - DNA, 21 bp, Artificial Sequence
  Primer
gattaggccaactgtggagca

SEQ ID NO: 69 - DNA, 26 bp, Artificial Sequence
  Primer
gcctctactcatcactacctgttttc

SEQ ID NO: 70 - DNA, 23 bp, Artificial Sequence
  Primer
tcagagagttcattttgctttcc

SEQ ID NO: 71 - DNA, 22 bp, Artificial Sequence
  Primer
cctcactacatccgtgaactcc

SEQ ID NO: 72 - DNA, 20 bp, Artificial Sequence
  Primer
ctgctggtatccttggcttc

SEQ ID NO: 73 - DNA, 19 bp, Artificial Sequence
  Primer
cccctggttgttgtagcag

SEQ ID NO: 74 - DNA, 20 bp, Artificial Sequence
  Primer
gtaggaggtgcgagttcagg

SEQ ID NO: 75 - DNA, 19 bp, Artificial Sequence
  Primer
cttcgactgcgtgctcaag

SEQ ID NO: 76 - DNA, 18 bp, Artificial Sequence
  Primer
gtaggtggcgaggggaag

SEQ ID NO: 77 - DNA, 20 bp, Artificial Sequence
  Primer
ggatctggcccttgaacctt

SEQ ID NO: 78 - DNA, 18 bp, Artificial Sequence
  Primer
gaaactggcggaaaccca

SEQ ID NO: 79 - protein, 283 aa, Homo sapiens
MEPPGDWGPPPWRSTPKTDVLRLVLYLTFLGAPCYAPALPSCKEDEYPVGSECCPKCSPGYRVKEACGELTGTVCEPCPPGTYIAHLNGLSKCLQCQMCDPAMGLRASRNCSRTENAVCGCSPGHFCIVQDGDHCAACRAYATSSPGQRVQKGGTESQDTLCQNCPPGTFSPNGTLEECQHQTKCSWLVTKAGAGTSSSHWVWWFLSGSLVIVIVCSTVGLIICVKRRKPRGDVVKVIVSVQRKRQEAEGEATVIEALQAPPDVTTVAVEETIPSFTGRSPNH

SEQ ID NO: 80 - protein, 78 aa, Homo sapiens
CKEDEYPVGSECCPKCSPGYRVKEACGELTGTVCEPCPPGTYIAHLNGLSKCLQCQMCDPAMGLRASRNCSRTENAVC

SEQ ID NO: 81 - protein, 73 aa, Human herpesvirus 5
CKPEEVQLGNQCCPPCKQGYRVTGQCTQYTSTTCTLCPNGTYVSGLYNCTNCTECNDTEVTIRNCTSTNNTVC

SEQ ID NO: 82 - protein, 78 aa, Artificial Sequence
  Synthetic construct: Consensus sequence
  MISC_FEATURE (3)..(3): Xaa is E or P
  MISC_FEATURE (4)..(4): Xaa is D or E
  MISC_FEATURE (6)..(6): Xaa is Y or V
  MISC_FEATURE (7)..(7): Xaa is P or Q
  MISC_FEATURE (8)..(8): Xaa is V or L
  MISC_FEATURE (10)..(10): Xaa is S or N
  MISC_FEATURE (11)..(11): Xaa is E or Q
  MISC_FEATURE (15)..(15): Xaa is K or P
  MISC_FEATURE (17)..(17): Xaa is S or K
  MISC_FEATURE (18)..(18): Xaa is P or Q
  MISC_FEATURE (23)..(23): Xaa is K or T
  MISC_FEATURE (24)..(24): Xaa is E or G
  MISC_FEATURE (25)..(25): Xaa is A or Q
  MISC_FEATURE (27)..(27): Xaa is G or T
  MISC_FEATURE (28)..(28): Xaa is E or Q
  MISC_FEATURE (29)..(29): Xaa is L or Y
  MISC_FEATURE (31)..(31): Xaa is G or S
  MISC_FEATURE (33)..(33): Xaa is V or T
  MISC_FEATURE (35)..(35): Xaa is E or T
  MISC_FEATURE (36)..(36): Xaa is P or L
  MISC_FEATURE (39)..(39): Xaa is P or N
  MISC_FEATURE (43)..(43): Xaa is I or V
  MISC_FEATURE (44)..(44): Xaa is A or S
  MISC_FEATURE (50)..(50): Xaa is S or Y
  MISC_FEATURE (51)..(51): Xaa is K or N
  MISC_FEATURE (53)..(53): Xaa is L or T
  MISC_FEATURE (54)..(54): Xaa is Q or N
  MISC_FEATURE (56)..(56): Xaa is Q or T
  MISC_FEATURE (57)..(57): Xaa is M or E
  MISC_FEATURE (59)..(59): Xaa is D or N
  MISC_FEATURE (60)..(60): Xaa is P or D
  MISC_FEATURE (61)..(61): Xaa is A or T
  MISC_FEATURE (62)..(62): Xaa is M or E
  MISC_FEATURE (65)..(65): Xaa is R or V
  MISC_FEATURE (66)..(66): Xaa is A or T
  MISC_FEATURE (67)..(67): Xaa is S or I
  MISC_FEATURE (71)..(71): Xaa is S or T
  MISC_FEATURE (72)..(72): Xaa is R or S
  MISC_FEATURE (74)..(74): Xaa is E or N
  MISC_FEATURE (76)..(76): Xaa is A or T
CKXXEXXXGXXCCPXCXXGYRVXXXCXXXTXTXCXXCPXGTYXXHLNGLXXCXXCXXCXXXXGLXXXRNCXXTXNXVC